European Patent Application EP 4 410 807 A1, published August 7, 2024. Title: Peptide Having Anti-Aging Activity and Uses Thereof. Applicant: CAREGEN CO., LTD. The sequence listing filed with the application follows.

SEQUENCE LISTING (13 sequences)

SEQ ID NO: 1 - protein, 7 aa, Artificial Sequence
  peptide
KRRRKRK

SEQ ID NO: 2 - DNA, 20 bp, Artificial Sequence
  Col1a1-F
caccctcaagagcctgagtc

SEQ ID NO: 3 - DNA, 20 bp, Artificial Sequence
  Col1a1-R
agacggctgagtagggaaca

SEQ ID NO: 4 - DNA, 20 bp, Artificial Sequence
  Fibronectin-F
ccaggaaccgagtacaccat

SEQ ID NO: 5 - DNA, 20 bp, Artificial Sequence
  Fibronectin-R
atacccaggttgggtgatga

SEQ ID NO: 6 - DNA, 20 bp, Artificial Sequence
  Elastin-F
gcaagacctggctttggact

SEQ ID NO: 7 - DNA, 21 bp, Artificial Sequence
  Elastin-R
gggagtttctggttagggctg

SEQ ID NO: 8 - DNA, 20 bp, Artificial Sequence
  SIRT1-F
tcagtggctggaacagtgag

SEQ ID NO: 9 - DNA, 20 bp, Artificial Sequence
  SIRT1-R
tctggcatgtcccactatca

SEQ ID NO: 10 - DNA, 20 bp, Artificial Sequence
  AQP3-F
ccttcttgggtgctggaata

SEQ ID NO: 11 - DNA, 20 bp, Artificial Sequence
  AQP3-R
acacgataagggaggctgtg

SEQ ID NO: 12 - DNA, 20 bp, Artificial Sequence
  GAPDH-F
ggagccaaaagggtcatcat

SEQ ID NO: 13 - DNA, 20 bp, Artificial Sequence
  GAPDH-R
gtgatggcatggactgtggt